European Patent Application EP 4 151 735 A1, published March 22, 2023. Title: VIRAL AND NON-VIRAL NANOPLASMID VECTORS WITH IMPROVED PRODUCTION. Applicant: NATURE TECHNOLOGY CORPORATION. Application US PCT/US2019/023209, filed March 20, 2019. The sequence listing filed with the application follows.

SEQUENCE LISTING (23 sequences)

SEQ ID NO: 1 - DNA, 281 bp, synthetic construct
  misc_feature 1..281: note = R6K gamma origin
  source 1..281: mol_type = other DNA
ggcttgttgtccacaaccgttaaaccttaaaagctttaaaagccttatatattcttttttttcttataaaacttaaaaccttagaggctatttaagttgctgatttatattaattttattgttcaaacatgagagcttagtacgtgaaacatgagagcttagtacgttagccatgagagcttagtacgttagccatgagggtttagttcgttaaacatgagagcttagtacgttaaacatgagagcttagtacgtactatcaacaggttgaactgctgatc

SEQ ID NO: 2 - DNA, 281 bp, synthetic construct
  misc_feature 1..281: note = 1 CpG R6K gamma origin
  source 1..281: mol_type = other DNA
ggcttgttgtccacaaccattaaaccttaaaagctttaaaagccttatatattcttttttttcttataaaacttaaaaccttagaggctatttaagttgctgatttatattaattttattgttcaaacatgagagcttagtacgtgaaacatgagagcttagtacattagccatgagagcttagtacattagccatgagggtttagttcattaaacatgagagcttagtacattaaacatgagagcttagtacatactatcaacaggttgaactgctgatc

SEQ ID NO: 3 - DNA, 260 bp, synthetic construct
  misc_feature 1..260: note = CpG free R6K gamma origin
  source 1..260: mol_type = other DNA
aaaccttaaaacctttaaaagccttatatattcttttttttcttataaaacttaaaaccttagaggctatttaagttgctgatttatattaattttattgttcaaacatgagagcttagtacatgaaacatgagagcttagtacattagccatgagagcttagtacattagccatgagggtttagttcattaaacatgagagcttagtacattaaacatgagagcttagtacatactatcaacaggttgaactgctgatc

SEQ ID NO: 4 - DNA, 389 bp, synthetic construct
  misc_feature 1..389: note = Extended R6K gamma origin
  source 1..389: mol_type = other DNA
tgtcagccgttaagtgttcctgtgtcactgaaaattgctttgagaggctctaagggcttctcagtgcgttacatccctggcttgttgtccacaaccgttaaaccttaaaagctttaaaagccttatatattcttttttttcttataaaacttaaaaccttagaggctatttaagttgctgatttatattaattttattgttcaaacatgagagcttagtacgtgaaacatgagagcttagtacgttagccatgagagcttagtacgttagccatgagggtttagttcgttaaacatgagagcttagtacgttaaacatgagagcttagtacgtgaaacatgagagcttagtacgtactatcaacaggttgaactgctgatcttcagatc

SEQ ID NO: 5 - DNA, 139 bp, synthetic construct
  misc_feature 1..139: note = RNA-OUT selectable marker
  source 1..139: mol_type = other DNA
gtagaattggtaaagagagtcgtgtaaaatatcgagttcgcacatcttgttgtctgattattgatttttggcgaaaccatttgatcatatgacaagatgtgtatctaccttaacttaatgattttgataaaaatcatta

SEQ ID NO: 6 - DNA, 69 bp, synthetic construct
  misc_feature 1..69: note = RNA-OUT antisense repressor RNA
  source 1..69: mol_type = other DNA
tcgcacatcttgttgtctgattattgatttttggcgaaaccatttgatcatatgacaagatgtgtatct

SEQ ID NO: 7 - DNA, 139 bp, synthetic construct
  misc_feature 1..139: note = 2 CpG RNA-OUT selectable marker
  source 1..139: mol_type = other DNA
gtagaattggtaaagagagttgtgtaaaatattgagttcgcacatcttgttgtctgattattgatttttggcgaaaccatttgatcatatgacaagatgtgtatctaccttaacttaatgattttgataaaaatcatta

SEQ ID NO: 8 - DNA, 466 bp, synthetic construct
  misc_feature 1..466: note = R6K gamma origin -RNA-OUT bacterial replication-selection regionflanked by NheI and KpnI restrictionsites
  source 1..466: mol_type = other DNA
gctagcccgcctaatgagcgggcttttttttggcttgttgtccacaaccgttaaaccttaaaagctttaaaagccttatatattcttttttttcttataaaacttaaaaccttagaggctatttaagttgctgatttatattaattttattgttcaaacatgagagcttagtacgtgaaacatgagagcttagtacgttagccatgagagcttagtacgttagccatgagggtttagttcgttaaacatgagagcttagtacgttaaacatgagagcttagtacgtactatcaacaggttgaactgctgatccacgttgtggtagaattggtaaagagagtcgtgtaaaatatcgagttcgcacatcttgttgtctgattattgatttttggcgaaaccatttgatcatatgacaagatgtgtatctaccttaacttaatgattttgataaaaatcattaggtacc

SEQ ID NO: 9 - DNA, 439 bp, synthetic construct
  misc_feature 1..439: note = 1 CpG R6K gamma origin - 2 CpG RNA-OUT bacterialreplication-selection region flanked by NheI and KpnI restrictionsites
  source 1..439: mol_type = other DNA
gctagctggcttgttgtccacaaccattaaaccttaaaagctttaaaagccttatatattcttttttttcttataaaacttaaaaccttagaggctatttaagttgctgatttatattaattttattgttcaaacatgagagcttagtacgtgaaacatgagagcttagtacattagccatgagagcttagtacattagccatgagggtttagttcattaaacatgagagcttagtacattaaacatgagagcttagtacatactatcaacaggttgaactgctgatctgtacagtagaattggtaaagagagttgtgtaaaatattgagttcgcacatcttgttgtctgattattgatttttggcgaaaccatttgatcatatgacaagatgtgtatctaccttaacttaatgattttgataaaaatcattaggtacc

SEQ ID NO: 10 - DNA, 565 bp, synthetic construct
  misc_feature 1..565: note = pNTC-NP1 polylinker trpA R6K-RNA-OUT polylinker cloning cassette:EcoRI-HindIII
  source 1..565: mol_type = other DNA
gaattcgagctcggtacctcgcgaatgcatctaggggacggccgctagcccgcctaatgagcgggcttttttttggcttgttgtccacaaccgttaaaccttaaaagctttaaaagccttatatattcttttttttcttataaaacttaaaaccttagaggctatttaagttgctgatttatattaattttattgttcaaacatgagagcttagtacgtgaaacatgagagcttagtacgttagccatgagagcttagtacgttagccatgagggtttagttcgttaaacatgagagcttagtacgttaaacatgagagcttagtacgtactatcaacaggttgaactgctgatccacgttgtggtagaattggtaaagagagtcgtgtaaaatatcgagttcgcacatcttgttgtctgattattgatttttggcgaaaccatttgatcatatgacaagatgtgtatctaccttaacttaatgattttgataaaaatcattaggagctagcattgggtcatcggatcccgggcccgtcgactgcagaggcctgcatgcaagctt

SEQ ID NO: 11 - DNA, 584 bp, synthetic construct
  misc_feature 1..584: note = pNTC-NP2 polylinker trpA R6K-RNA-OUTpolylinker cloningcassette: EcoRI-HindIII
  source 1..584: mol_type = other DNA
gaattcgagctcggtacctcgcgaatgcatctaggggacggccgctagcccgcctaatgagcgggcttttttttggcttgttgtccacaaccgttaaaccttaaaagctttaaaagccttatatattcttttttttcttataaaacttaaaaccttagaggctatttaagttgctgatttatattaattttattgttcaaacatgagagcttagtacgtgaaacatgagagcttagtacgttagccatgagagcttagtacgttagccatgagggtttagttcgttaaacatgagagcttagtacgttaaacatgagagcttagtacgtactatcaacaggttgaactgctgatccacgttgtggtagaattggtaaagagagtcgtgtaaaatatcgagttcgcacatcttgttgtctgattattgatttttggcgaaaccatttgatcatatgacaagatgtgtatctaccttaacttaatgattttgataaaaatcattaggactagtcccgggcgctagttattaatattgggtcatcggatcccgggcccgtcgactgcagaggcctgcatgcaagctt

SEQ ID NO: 12 - DNA, 557 bp, synthetic construct
  misc_feature 1..557: note = pNTC-NP3 polylinker trpA R6K-RNA-OUTpolylinker cloningcassette: EcoRI-HindIII
  source 1..557: mol_type = other DNA
gaattcgagctcggtacctcgcgaatgcatctaggggacggccgctagcccgcctaatgagcgggcttttttttggcttgttgtccacaaccgttaaaccttaaaagctttaaaagccttatatattcttttttttcttataaaacttaaaaccttagaggctatttaagttgctgatttatattaattttattgttcaaacatgagagcttagtacgtgaaacatgagagcttagtacgttagccatgagagcttagtacgttagccatgagggtttagttcgttaaacatgagagcttagtacgttaaacatgagagcttagtacgtactatcaacaggttgaactgctgatccacgttgtggtagaattggtaaagagagtcgtgtaaaatatcgagttcgcacatcttgttgtctgattattgatttttggcgaaaccatttgatcatatgacaagatgtgtatctaccttaacttaatgattttgataaaaatcattaggtaccgagctcggatcccgggcccgtcgactgcagaggcctgcatgcaagctt

SEQ ID NO: 13 - DNA, 557 bp, synthetic construct
  misc_feature 1..557: note = pNTC-NP4 polylinker trpA R6K-RNA-OUTpolylinker cloningcassette: HindIII-EcoRI
  source 1..557: mol_type = other DNA
aagcttgcatgcaggcctctgcagtcgacgggcccgggatccgagctcggtacctcgcgaatgcatctaggggacggccgctagcccgcctaatgagcgggcttttttttggcttgttgtccacaaccgttaaaccttaaaagctttaaaagccttatatattcttttttttcttataaaacttaaaaccttagaggctatttaagttgctgatttatattaattttattgttcaaacatgagagcttagtacgtgaaacatgagagcttagtacgttagccatgagagcttagtacgttagccatgagggtttagttcgttaaacatgagagcttagtacgttaaacatgagagcttagtacgtactatcaacaggttgaactgctgatccacgttgtggtagaattggtaaagagagtcgtgtaaaatatcgagttcgcacatcttgttgtctgattattgatttttggcgaaaccatttgatcatatgacaagatgtgtatctaccttaacttaatgattttgataaaaatcattaggtaccgagctcgaattc

SEQ ID NO: 14 - DNA, 503 bp, synthetic construct
  misc_feature 1..503: note = pNTC-NP5 polylinker trpA R6K-RNA-OUTpolylinker cloningcassette: KasI-HindIII
  source 1..503: mol_type = other DNA
ggcgccgctagcccgcctaatgagcgggcttttttttggcttgttgtccacaaccgttaaaccttaaaagctttaaaagccttatatattcttttttttcttataaaacttaaaaccttagaggctatttaagttgctgatttatattaattttattgttcaaacatgagagcttagtacgtgaaacatgagagcttagtacgttagccatgagagcttagtacgttagccatgagggtttagttcgttaaacatgagagcttagtacgttaaacatgagagcttagtacgtactatcaacaggttgaactgctgatccacgttgtggtagaattggtaaagagagtcgtgtaaaatatcgagttcgcacatcttgttgtctgattattgatttttggcgaaaccatttgatcatatgacaagatgtgtatctaccttaacttaatgattttgataaaaatcattaggtaccacatgtcctgcagaggcctgcatgcaagctt

SEQ ID NO: 15 - DNA, 539 bp, synthetic construct
  misc_feature 1..539: note = pNTC-NP6 polylinker trpA R6K-RNA-OUTpolylinker cloningcassette: EcoRI-SacI
  source 1..539: mol_type = other DNA
gaattctgcagatatccatcacactggcggccgctagcccgcctaatgagcgggcttttttttggcttgttgtccacaaccgttaaaccttaaaagctttaaaagccttatatattcttttttttcttataaaacttaaaaccttagaggctatttaagttgctgatttatattaattttattgttcaaacatgagagcttagtacgtgaaacatgagagcttagtacgttagccatgagagcttagtacgttagccatgagggtttagttcgttaaacatgagagcttagtacgttaaacatgagagcttagtacgtactatcaacaggttgaactgctgatccacgttgtggtagaattggtaaagagagtcgtgtaaaatatcgagttcgcacatcttgttgtctgattattgatttttggcgaaaccatttgatcatatgacaagatgtgtatctaccttaacttaatgattttgataaaaatcattaggtaccgggccccccctcgatcgaggtcgacggtatcgggggagctc

SEQ ID NO: 16 - DNA, 500 bp, synthetic construct
  misc_feature 1..500: note = pNTC-NP7 polylinker trpA R6K-RNA-OUTpolylinker cloningcassette: BssHII-BssHII
  source 1..500: mol_type = other DNA
gcgcgcagccttaattaagctagcccgcctaatgagcgggcttttttttggcttgttgtccacaaccgttaaaccttaaaagctttaaaagccttatatattcttttttttcttataaaacttaaaaccttagaggctatttaagttgctgatttatattaattttattgttcaaacatgagagcttagtacgtgaaacatgagagcttagtacgttagccatgagagcttagtacgttagccatgagggtttagttcgttaaacatgagagcttagtacgttaaacatgagagcttagtacgtactatcaacaggttgaactgctgatccacgttgtggtagaattggtaaagagagtcgtgtaaaatatcgagttcgcacatcttgttgtctgattattgatttttggcgaaaccatttgatcatatgacaagatgtgtatctaccttaacttaatgattttgataaaaatcattaggtaccttaattaactgcgcgc

SEQ ID NO: 17 - DNA, 530 bp, synthetic construct
  misc_feature 1..530: note = pNTC-3xCpG NP1 polylinker R6K-RNA-OUTpolylinker cloningcassette: HindIII-EcoRI
  source 1..530: mol_type = other DNA
aagcttgcatgcaggcctctgcagtcgacgggccctctagactcgagctggcttgttgtccacaaccattaaaccttaaaagctttaaaagccttatatattcttttttttcttataaaacttaaaaccttagaggctatttaagttgctgatttatattaattttattgttcaaacatgagagcttagtacgtgaaacatgagagcttagtacattagccatgagagcttagtacattagccatgagggtttagttcattaaacatgagagcttagtacattaaacatgagagcttagtacatactatcaacaggttgaactgctgatctgtacagtagaattggtaaagagagttgtgtaaaatattgagttcgcacatcttgttgtctgattattgatttttggcgaaaccatttgatcatatgacaagatgtgtatctaccttaacttaatgattttgataaaaatcattaggtaccgctagcggccgtcccctagatgcattcgcgaggtaccgagctcgaattc

SEQ ID NO: 18 - DNA, 303 bp, synthetic construct
  misc_feature 1..303: note = R6K gamma origin -7 iteron
  source 1..303: mol_type = other DNA
ggcttgttgtccacaaccgttaaaccttaaaagctttaaaagccttatatattcttttttttcttataaaacttaaaaccttagaggctatttaagttgctgatttatattaattttattgttcaaacatgagagcttagtacgtgaaacatgagagcttagtacgttagccatgagagcttagtacgttagccatgagggtttagttcgttaaacatgagagcttagtacgttaaacatgagagcttagtacgttaaacatgagagcttagtacgtactatcaacaggttgaactgctgatc

SEQ ID NO: 19 - DNA, 22 bp, synthetic construct
  misc_feature 1..22: note = R6K gamma origin iteron
  source 1..22: mol_type = other DNA
aaacatgagagcttagtacgtg

SEQ ID NO: 20 - DNA, 22 bp, synthetic construct
  misc_feature 1..22: note = R6K gamma origin iteron
  source 1..22: mol_type = other DNA
aaacatgagagcttagtacgtt

SEQ ID NO: 21 - DNA, 22 bp, synthetic construct
  misc_feature 1..22: note = R6K gamma origin iteron
  source 1..22: mol_type = other DNA
agccatgagagcttagtacgtt

SEQ ID NO: 22 - DNA, 22 bp, synthetic construct
  misc_feature 1..22: note = R6K gamma origin iteron
  source 1..22: mol_type = other DNA
agccatgagggtttagttcgtt

SEQ ID NO: 23 - DNA, 22 bp, synthetic construct
  misc_feature 1..22: note = R6K gamma origin iteron
  source 1..22: mol_type = other DNA
aaacatgagagcttagtacgta